European Patent Specification EP 3 839 041 B1, published August 5, 2026. Title: Semi-Continuous Culture Methods. Applicant: Mara Renewables Corporation. The sequence listing filed with the application follows.

SEQUENCE LISTING (1 sequence)

SEQ ID NO: 1 - DNA, 1723 bp, Artificial Sequence
  Synthetic Construct
gtagtcatacgctcgtctcaaagattaagccatgcatgtgtaagtataagcgattatactgtgagactgcgaacggctcattatatcagttatgatttcttcggtattttctttatatggatacctgcagtaattctggaattaatacatgctgagagggcccgactgttcgggagggccgcacttattagagttgaagccaagtaagatggtgagtcatgataattgagcagatcgcttgtttggagcgatgaatcgtttgagtttctgccccatcagttgtcgacggtagtgtattggactacggtgactataacgggtgacggggagttagggctcgactccggagagggagcctgagagacggctaccacatccaaggaaggcagcaggcgcgtaaattacccaatgtggactccacgaggtagtgacgagaaatatcaatgcggggcgcttcgcgtcttgctattggaatgagagcaatgtaaaaccctcatcgaggatcaactggagggcaagtctggtgccagcagccgcggtaattccagctccagaagcgtatgctaaagttgttgcagttaaaaagctcgtagttgaatttctggggcgggagccccggtctttgcgcgactgcgctctgtttgccgagcggctcctctgccatcctcgcctctttttttagtggcgtcgttcactgtaattaaagcagagtgttccaagcaggtcgtatgacctggatgtttattatgggatgatcagatagggctcgggtgctattttgttggtttgcacatctgagtaatgatgaataggaacagttgggggtattcgtatttaggagctagaggtgaaattcttggatttccgaaagacgaactacagcgaaggcatttaccaagcatgttttcattaatcaagaacgaaagtctggggatcgaagatgattagataccatcgtagtctagaccgtaaacgatgccgacttgcgattgcggggtgtttgtattggaccctcgcagcagcacatgagaaatcaaagtctttgggttccggggggagtatggtcgcaaggctgaaacttaaaggaattgacggaagggcaccaccaggagtggagcctgcggcttaatttgactcaacacgggaaaacttaccaggtccagacataggtaggattgacagattgagagctctttcttgattctatgggtggtggtgcatggccgttcttagttggtggagtgatttgtctggttaattccgttaacgaacgagacctcggcctactaaatagcggtgggtatggcgacatacttgcgtacgcttcttagagggacatgttcggtatacgagcaggaagttcgaggcaataacaggtctgtgatgcccttagatgttctgggccgcacgcgcgctacactgatgggttcaacgggtggtcatcgttgttcgcagcgaggtgctttgccggaaggcatggcaaatcctttcaacgcccatcgtgctggggctagatttttgcaattattaatctccaacgaggaattcctagtaaacgcaagtcatcagcttgcattgaatacgtccctgccctttgtacacaccgcccgtcgcacctaccgattgaacggtccgatgaaaccatgggatgaccttttgagcgtttgttcgcgaggggggtcagaactcgggtgaatcttattgtttagaggaaggtgaagtc